European Patent Application EP 4 349 977 A1, published April 10, 2024. Title: 耐热B家族DNA聚合酶突变体及其应用. Applicant: 深圳华大生命科学研究院. The sequence listing filed with the application follows.

SEQUENCE LISTING (5 sequences)

SEQ ID NO: 1 - protein, 774 aa, Artificial sequence
MILDTDYITEDGKPVIRIFKKENGEFKIEYDRTFEPYFYALLKDDSAIEEVKKITAERHGTVVTVKRVEKVQKKFLGRPVEVWKLYFTHPQDVPAIRDKIREHPAVIDIYEYDIPFAKRYLIDKGLVPMEGDEELKMLAFAIATLYHEGEEFAEGPILMISYADEEGARVITWKNVDLPYVDVVSTEREMIKRFLRVVKEKDPDVLITYNGDNFDFAYLKKRCEKLGINFALGRDGSEPKIQRMGDRFAVEVKGRIHFDLYPVIRRTINLPTYTLEAVYEAVFGQPKEKVYAEEITTAWETGENLERVARYSMEDAKVTYELGKEFLPMEAQLSRLIGQSLWDVSRSSTGNLVEWFLLRKAYERNELAPNKPDEKELARRRQSYEGGYVKEPERGLWENIVYLDFRSLYPSIIITHNVSPDTLNREGCKEYDVAPQVGHRFCKDFPGFIPSLLGDLLEERQKIKKKMKATIDPIERKLLDYRQRAIKILANSYYGYYGYARARWYCKECAESVTAWGREYITMTIKEIEEKYGFKVIYSDTDGFFATIPGADAETVKKKAMEFLKYINAKLPGALELEYEGFYKRGFFVTKKKYAVIDEEGKITTRGLEIVRRDWSEIAKETQARVLEALLKDGDVEKAVRIVKEVTEKLSKYEVPPEKLVIHEQITRDLKDYKATGPHVAVAKRLAARGVKIRPGTVISYIVLKGSGRIGDRAIPFDEFDPTKHKYDAEYYIENQVLPAVERILRAFGYRKEDLRYQKTRQVGLSAWLKPKGT

SEQ ID NO: 2 - protein, 775 aa, Artificial sequence
MILDTDYITENGKPVIRVFKKENGEFKIEYDRTFEPYFYALLKDDSAIEDVKKVTAKRHGTVVKVKRAEKVQKKFLGRPIEVWKLYFNHPQDVPAIRDRIRAHPAVVDIYEYDIPFAKRYLIDKGLIPMEGDEELTMLAFAIATLYHEGEEFGTGPILMISYADGSEARVITWKKIDLPYVDVVSTEKEMIKRFLRVVREKDPDVLITYNGDNFDFAYLKKRCEELGIKFTLGRDGSEPKIQRMGDRFAVEVKGRIHFDLYPVIRRTINLPTYTLEAVYEAVFGKPKEKVYAEEIAQAWESGEGLERVARYSMEDAKVTYELGREFFPMEAQLSRLIGQSLWDVSRSSTGNLVEWFLLRKAYKRNELAPNKPDERELARRRGGYAGGYVKEPERGLWDNIVYLDFRSLYPSIIITHNVSPDTLNREGCKEYDVAPEVGHKFCKDFPGFIPSLLGDLLEERQKIKRKMKATVDPLEKKLLDYRQRAIKILANSFYGYYGYAKARWYCKECAESVTAWGREYIEMVIRELEEKFGFKVLYADTDGLHATIPGADAETVKKKAKEFLKYINPKLPGLLELEYEGFYVRGFFVTKKKYAVIDEEGKITTRGLEIVRRDWSEIAKETQARVLEAILKHGDVEEAVRIVKEVTEKLSKYEVPPEKLVIHEQITRDLRDYKATGPHVAVAKRLAARGVKIRPGTVISYIVLKGSGRIGDRAIPADEFDPTKHRYDAEYYIENQVLPAVERILKAFGYRKEDLRYQKTKQVGLGAWLKVKGKK

SEQ ID NO: 3 - protein, 773 aa, Artificial sequence
MILDTDYITEDGKPVIRIFKKENGEFKIDYDRNFEPYIYALLKDDSAIEDVKKITAERHGTTVRVVRAEKVKKKFLGRPIEVWKLYFTHPQDVPAIRDKIKEHPAVVDIYEYDIPFAKRYLIDKGLIPMEGDEELKMLAFAIATLYHEGEEFAEGPILMISYADEEGARVITWKNIDLPYVDVVSTEKEMIKRFLKVVKEKDPDVLITYNGDNFDFAYLKKRSEKLGVKFILGREGSEPKIQRMGDRFAVEVKGRIHFDLYPVIRRTINLPTYTLEAVYEAIFGQPKEKVYAEEIAQAWETGEGLERVARYSMEDAKVTYELGKEFFPMEAQLSRLVGQSLWDVSRSSTGNLVEWFLLRKAYERNELAPNKPDERELARRRESYAGGYVKEPERGLWENIVYLDFRSLYPSIIITHNVSPDTLNREGCEEYDVAPQVGHKFCKDFPGFIPSLLGDLLEERQKVKKKMKATIDPIEKKLLDYRQRAIKILANSFYGYYGYAKARWYCKECAESVTAWGRQYIETTIREIEEKFGFKVLYADTDGFFATIPGADAETVKKKAKEFLDYINAKLPGLLELEYEGFYKRGFFVTKKKYAVIDEEDKITTRGLEIVRRDWSEIAKETQARVLEAILKHGDVEEAVRIVKEVTEKLSKYEVPPEKLVIYEQITRDLKDYKATGPHVAVAKRLAARGIKIRPGTVISYIVLKGSGRIGDRAIPFDEFDPAKHKYDAEYYIENQVLPAVERILRAFGYRKEDLRYQKTRQVGLGAWLKPKT

SEQ ID NO: 4 - protein, 773 aa, Artificial sequence
MILDADYITEDGKPVIRVFKKEKGEFKIDYDRDFEPYIYALLKDDSAIEDIKKITAERHGTTVRVTRAERVKKKFLGRPVEVWKLYFTHPQDVPAIRDKIREHPAVVDIYEYDIPFAKRYLIDRGLIPMEGDEELRMLAFAIATLYHEGEEFGEGPILMISYADEEGARVITWKNIDLPYVESVSTEKEMIKRFLKVIQEKDPDVLITYNGDNFDFAYLKKRSEMLGVKFILGRDGSEPKIQRMGDRFAVEVKGRIHFDLYPVIRRTINLPTYTLETVYEPVFGQPKEKVYAEEIARAWESGEGLERVARYSMEDAKATYELGKEFFPMEAQLSRLVGQSLWDVSRSSTGNLVEWFLLRKAYERNDVAPNKPDERELARRTESYAGGYVKEPEKGLWENIVYLDYKSLYPSIIITHNVSPDTLNREGCREYDVAPQVGHRFCKDFPGFIPSLLGDLLEERQKVKKKMKATVDPIERKLLDYRQRAIKILANSYYGYYAYANARWYCRECAESVTAWGRQYIETTMREIEEKFGFKVLYADTDGFFATIPGADAETVKNKAKEFLNYINPRLPGLLELEYEGFYRRGFFVTKKKYAVIDEEDKITTRGLEIVRRDWSEIAKETQARVLEAILKHGDVEEAVRIVKEVTEKLSRHEVPPEKLVIYEQITRDLRSYRATGPHVAVAKRLAARGIKIRPGTVISYIVLKGPGRVGDRAIPFDEFDPAKHRYDAEYYIENQVLPAVERILRAFGYRKEDLRYQKTKQAGLGAWLKPKT

SEQ ID NO: 5 - protein, 774 aa, Artificial sequence
MILDTDYITEDGKPVIRIFKKENGEFKIEYDRTFEPYFYALLKDDSAIEEVKKITAERHGTVVTVKRVEKVQKKFLGRPVEVWKLYFTHPQDVPAIRDKIREHPAVIDIYEYDIPFAKRYLIDKGLVPMEGDEELKMLAFAIATLYHEGEEFAEGPILMISYADEEGARVITWKNVDLPYVDVVSTEREMIKRFLRVVKEKDPDVLITYNGDNFDFAYLKKRCEKLGINFALGRDGSEPKIQRMGDRFAVEVKGRIHFDLYPVIRRTINLPTYTLEAVYEAVFGQPKEKVYAEEITTAWETGENLERVARYSMEDAKVTYELGKEFLPMEAQLSRLIGQSLWDVSRSSTGNLVEWFLLRKAYERNELAPNKPDEKELARRRQTFEGGYIKEPERGLWENIVYLDFRSIAPSIIITHNVSPDTLNREGCKEYDVAPQVGHRFCKDFPGFIPSLLGDLLEERQKIKKKMKATIDPIERKLLDYRQREIKILANSYYGYYGYARARWYCKECAESVTAWGREYITMTIKEIEEKYGFKVIYSDTDGFFATIPGADAETVKKKAMEFLKYINAKLPGALELEYEGFYKRGFFHTKKKYAVIDEEGKITTRGLEIVRRDWSEIAKETQARVLEALLKDGDVEKAVRIVKEVTEKLSKYEVPPEKLVIHEQITRDLKDYKAKGPHMAVAKRLAARGVKIRPGTVISYIVLKGSGRIGDRAIPFDEFDPTKHKYDAEYYIENQVLPAVERILRAFGYRKEDLRYQKTRQVGLSAWLKPKGT